European Patent Specification EP 3 781 589 B1, published October 4, 2023. Title: Means and methods for the treatment of Angiogenesis-, Fibrosis- and Cancer-related Diseases with protein oligomers comprising NC-1-Fc. Applicant: Universität Heidelberg. The sequence listing filed with the application follows.

SEQUENCE LISTING (42 sequences)

SEQ ID NO: 1 - protein, 1527 aa, Mus musculus
MAPDPSRRLCLLLLLLLSCRLVPASADGNSLSPLNPLVWLWPPKTSDSLEGPVSKPQNSSPVQSTENPTTHVVPQDGLTEQQTTPASSELPPEEEEEEDQKAGQGGSPATPAVPIPLVAPAASPDMKEENVAGVGAKILNVAQGIRSFVQLWDEDSTIGHSAGTEVPDSSIPTVLPSPAELSSAPQGSKTTLWLSSAIPSSPDAQTTEAGTLAVPTQLPPFQSNLQAPLGRPSAPPDFPENVAEEVGLLQLLGDPLPEKISQIDDPHVGPAYIFGPDSNSGQVAQYHFPKLFFRDFSLLFHVRPATEAAGVLFAITDAAQVVVSLGVKLSEVRDGQQNISLLYTEPGASQTQTGASFRLPAFVGQWTHFALSVDGGSVALYVDCEEFQRVPFARASQGLELERGAGLFVGQAGTADPDKFQGMISELKVRKTPRVSPVHCLDEEDDDEDRASGDFGSGFEESSKSHKEDTSLLPGLPQPPPVTSPPLAGGSTTEDPRTEETEEDAAVDSIGAETLPGTGSSGAWDEAIQNPGRGLIKGGMKGQKGEPGAQGPPGPAGPQGPAGPVVQSPNSQPVPGAQGPPGPQGPPGKDGTPGRDGEPGDPGEDGRPGDTGPQGFPGTPGDVGPKGEKGDPGIGPRGPPGPPGPPGPSFRQDKLTFIDMEGSGFSGDIESLRGPRGFPGPPGPPGVPGLPGEPGRFGINGSYAPGPAGLPGVPGKEGPPGFPGPPGPPGPPGKEGPPGVAGQKGSVGDVGIPGPKGSKGDLGPIGMPGKSGLAGSPGPVGPPGPPGPPGPPGPGFAAGFDDMEGSGIPLWTTARSSDGLQGPPGSPGLKGDPGVAGLPGAKGEVGADGAQGIPGPPGREGAAGSPGPKGEKGMPGEKGNPGKDGVGRPGLPGPPGPPGPVIYVSSEDKAIVSTPGPEGKPGYAGFPGPAGPKGDLGSKGEQGLPGPKGEKGEPGTIFSPDGRALGHPQKGAKGEPGFRGPPGPYGRPGHKGEIGFPGRPGRPGTNGLKGEKGEPGDASLGFSMRGLPGPPGPPGPPGPPGMPIYDSNAFVESGRPGLPGQQGVQGPSGPKGDKGEVGPPGPPGQFPIDLFHLEAEMKGDKGDRGDAGQKGERGEPGAPGGGFFSSSVPGPPGPPGYPGIPGPKGESIRGPPGPPGPQGPPGIGYEGRQGPPGPPGPPGPPSFPGPHRQTVSVPGPPGPPGPPGPPGAMGASAGQVRIWATYQTMLDKIREVPEGWLIFVAEREELYVRVRNGFRKVLLEARTALPRGTGNEVAALQPPLVQLHEGSPYTRREYSYSTARPWRADDILANPPRLPDRQPYPGVPHHHSSYVHLPPARPTLSLAHTHQDFQPVLHLVALNTPLSGGMRGIRGADFQCFQQARAVGLSGTFRAFLSSRLQDLYSIVRRADRGSVPIVNLKDEVLSPSWDSLFSGSQGQLQPGARIFSFDGRDVLRHPAWPQKSVWHGSDPSGRRLMESYCETWRTETTGATGQASSLLSGRLLEQKAASCHNSYIVLCIENSFMTSFSK

SEQ ID NO: 2 - protein, 1516 aa, Homo sapiens
MAPYPCGCHILLLLFCCLAAARANLLNLNWLWFNNEDTSHAATTIPEPQGPLPVQPTADTTTHVTPRNGSTEPATAPGSPEPPSELLEDGQDTPTSAESPDAPEENIAGVGAEILNVAKGIRSFVQLWNDTVPTESLARAETLVLETPVGPLALAGPSSTPQENGTTLWPSRGIPSSPGAHTTEAGTLPAPTPSPPSLGRPWAPLTGPSVPPPSSERISEEVGLLQLLGDPPPQQVTQTDDPDVGLAYVFGPDANSGQVARYHFPSLFFRDFSLLFHIRPATEGPGVLFAITDSAQAMVLLGVKLSGVQDGHQDISLLYTEPGAGQTHTAASFRLPAFVGQWTHLALSVAGGFVALYVDCEEFQRMPLARSSRGLELEPGAGLFVAQAGGADPDKFQGVIAELKVRRDPQVSPMHCLDEEGDDSDGASGDSGSGLGDARELLREETGAALKPRLPAPPPVTTPPLAGGSSTEDSRSEEVEEQTTVASLGAQTLPGSDSVSTWDGSVRTPGGRVKEGGLKGQKGEPGVPGPPGRAGPPGSPCLPGPPGLPCPVSPLGPAGPALQTVPGPQGPPGPPGRDGTPGRDGEPGDPGEDGKPGDTGPQGFPGTPGDVGPKGDKGDPGVGERGPPGPQGPPGPPGPSFRHDKLTFIDMEGSGFGGDLEALRGPRGFPGPPGPPGVPGLPGEPGRFGVNSSDVPGPAGLPGVPGREGPPGFPGLPGPPGPPGREGPPGRTGQKGSLGEAGAPGHKGSKGAPGPAGARGESGLAGAPGPAGPPGPPGPPGPPGPGLPAGFDDMEGSGGPFWSTARSADGPQGPPGLPGLKGDPGVPGLPGAKGEVGADGVPGFPGLPGREGIAGPQGPKGDRGSRGEKGDPGKDGVGQPGLPGPPGPPGPVVYVSEQDGSVLSVPGPEGRPGFAGFPGPAGPKGNLGSKGERGSPGPKGEKGEPGSIFSPDGGALGPAQKGAKGEPGFRGPPGPYGRPGYKGEIGFPGRPGRPGMNGLKGEKGEPGDASLGFGMRGMPGPPGPPGPPGPPGTPVYDSNVFAESSRPGPPGLPGNQGPPGPKGAKGEVGPPGPPGQFPFDFLQLEAEMKGEKGDRGDAGQKGERGEPGGGGFFGSSLPGPPGPPGPRGYPGIPGPKGESIRGQPGPPGPQGPPGIGYEGRQGPPGPPGPPGPPSFPGPHRQTISVPGPPGPPGPPGPPGTMGASSGVRLWATRQAMLGQVHEVPEGWLIFVAEQEELYVRVQNGFRKVQLEARTPLPRGTDNEVAALQPPVVQLHDSNPYPRREHPHPTARPWRADDILASPPRLPEPQPYPGAPHHSSYVHLRPARPTSPPAHSHRDFQPVLHLVALNSPLSGGMRGIRGADFQCFQQARAVGLAGTFRAFLSSRLQDLYSIVRRADRAAVPIVNLKDELLFPSWEALFSGSEGPLKPGARIFSFDGKDVLRHPTWPQKSVWHGSDPNGRRLTESYCETWRTEAPSATGQASSLLGGRLLGQSAASCHHAYIVLCIENSFMTASK

SEQ ID NO: 3 - protein, 315 aa, Mus musculus
AGQVRIWATYQTMLDKIREVPEGWLIFVAEREELYVRVRNGFRKVLLEARTALPRGTGNEVAALQPPLVQLHEGSPYTRREYSYSTARPWRADDILANPPRLPDRQPYPGVPHHHSSYVHLPPARPTLSLAHTHQDFQPVLHLVALNTPLSGGMRGIRGADFQCFQQARAVGLSGTFRAFLSSRLQDLYSIVRRADRGSVPIVNLKDEVLSPSWDSLFSGSQGQLQPGARIFSFDGRDVLRHPAWPQKSVWHGSDPSGRRLMESYCETWRTETTGATGQASSLLSGRLLEQKAASCHNSYIVLCIENSFMTSFSK

SEQ ID NO: 4 - protein, 312 aa, Homo sapiens
SGVRLWATRQAMLGQVHEVPEGWLIFVAEQEELYVRVQNGFRKVQLEARTPLPRGTDNEVAALQPPVVQLHDSNPYPRREHPHPTARPWRADDILASPPRLPEPQPYPGAPHHSSYVHLRPARPTSPPAHSHRDFQPVLHLVALNSPLSGGMRGIRGADFQCFQQARAVGLAGTFRAFLSSRLQDLYSIVRRADRAAVPIVNLKDELLFPSWEALFSGSEGPLKPGARIFSFDGKDVLRHPTWPQKSVWHGSDPNGRRLTESYCETWRTEAPSATGQASSLLGGRLLGQSAASCHHAYIVLCIENSFMTASK

SEQ ID NO: 5 - protein, 233 aa, Mus musculus
EPRGPTIKPCPPCKCPAPNLLGGPSVFIFPPKIKDVLMISLSPIVTCVVVDVSEDDPDVQISWFVNNVEVHTAQTQTHREDYNSTLRVVSALPIQHQDWMSGKEFKCKVNNKDLPAPIERTISKPKGSVRAPQVYVLPPPEEEMTKKQVTLTCMVTDFMPEDIYVEWTNNGKTELNYKNTEPVLDSDGSYFMYSKLRVEKKNWVERNSYSCSVVHEGLHNHHTTKSFSRTPGK

SEQ ID NO: 6 - protein, 232 aa, Homo sapiens
EPKSSDKTHTCPPCPAPELLGGPSVFLFPPKPKDTLMISRTPEVTCVVVDVSHEDPEVKFNWYVDGVEVHNAKTKPREEQYNSTYRVVSVLTVLHQDWLNGKEYKCKVSNKALPAPIEKTISKAKGQPREPQVYTLPPSREEMTKNQVSLTCLVKGFYPSDIAVEWESNGQPENNYKTTPPVLDSDGSFFLYSKLTVDKSRWQQGNVFSCSVMHEALHNHYTQKSLSLSPGK

SEQ ID NO: 7 - protein, 28 aa, Mus musculus
HTHQDFQPVLHLVLYAVTGRGDSPASSK

SEQ ID NO: 8 - protein, 15 aa, Mus musculus
LYAVTGRGDSPASSK

SEQ ID NO: 9 - protein, 26 aa, Mus musculus
HTHQDFQPVLHLVALNTPLSGGMRGI

SEQ ID NO: 10 - protein, 25 aa, Homo sapiens
HSHRDFQPVLHLVALNSPLSGGMRG

SEQ ID NO: 11 - protein, 15 aa, Mus musculus
LYAVTGRGDSPASSK

SEQ ID NO: 12 - protein, 15 aa, Homo sapiens
VYAVTGRGDSPASSK

SEQ ID NO: 13 - protein, 27 aa, Homo sapiens
HSHRDFQPVLHLVYAVTGRGDSPASSK

SEQ ID NO: 14 - protein, 27 aa, Homo sapiens
ASARDFQPVLHLVYAVTGRGDSPASSK

SEQ ID NO: 15 - protein, 27 aa, Homo sapiens
HSHRDFCPVLHLVYAVTGRGDSPASSK

SEQ ID NO: 16 - protein, 27 aa, Homo sapiens
HSHRDFQPVLHLVYAVTGRADSPASSK

SEQ ID NO: 17 - protein, 25 aa, Mus musculus
IKPGADYTITLYAVTGRGDSPASSK

SEQ ID NO: 18 - protein, 184 aa, Mus musculus
HTHQDFQPVLHLVALNTPLSGGMRGIRGADFQCFQQARAVGLSGTFRAFLSSRLQDLYSIVRRADRGSVPIVNLKDEVLSPSWDSLFSGSQGQLQPGARIFSFDGRDVLRHPAWPQKSVWHGSDPSGRRLMESYCETWRTETTGATGQASSLLSGRLLEQKAASCHNSYIVLCIENSFMTSFSK

SEQ ID NO: 19 - protein, 180 aa, Homo sapiens
HSHRDFQPVLHLVALNAPLSGGMRGIRGADFQCFQQARAVGLAGTFRAFLSSRLQDLYSIVRRADRAAVPIVNLKDELLFPSWEALFSGSEGPLKPGARIFSFDGKDVLRHPTWPQKSVWHGSDPNGRRLTESYCETWRTEAPSATGQASSLLGGRLLGQSAASCHHAYIVLCIENSFMT

SEQ ID NO: 20 - protein, 27 aa, Mus musculus
HTHQDFQPVLHLVALNTPLSGGMRGIR

SEQ ID NO: 21 - protein, 48 aa, Homo sapiens
SYCETWRTEAPSATGQASSLLGGRLLGQSAASCHHAYIVLCIENSFMT

SEQ ID NO: 22 - protein, 27 aa, Homo sapiens
HSHRDFQPVLHLVALNAPLSGGMRGIR

SEQ ID NO: 23 - protein, 5 aa, Artificial Sequence
  Enterokinase cleavage site
DDDDK

SEQ ID NO: 24 - protein, 227 aa, Homo sapiens
DKTHTCPPCPAPELLGGPSVFLFPPKPKDTLMISRTPEVTCVVVDVSHEDPEVKFNWYVDGVEVHNAKTKPREEQYNSTYRVVSVLTVLHQDWLNGKEYKCKVSNKALPAPIEKTISKAKGQPREPQVYTLPPSRDELTKNQVSLTCLVKGFYPSDIAVEWESNGQPENNYKTTPPVLDSDGSFFLYSKLTVDKSRWQQGNVFSCSVMHEALHNHYTQKSLSLSPGK

SEQ ID NO: 25 - protein, 227 aa, Homo sapiens
DKTHTCPPCPAPELLGGPSVFLFPPKPKDTLMISRTPEVTCVVVDVSHEDPEVKFNWYVDGVEVHNAKTKPREEQYNSTYRVVSVLTVLHQDWLNGKEYKCKVSNKALPAPIEKTISKAKGQPREPQVYTLPPCRDELTKNQVSLWCLVKGFYPSDIAVEWESNGQPENNYKTTPPVLDSDGSFFLYSKLTVDKSRWQQGNVFSCSVMHEALHNHYTQKSLSLSPGK

SEQ ID NO: 26 - protein, 227 aa, Homo sapiens
DKTHTCPPCPAPELLGGPSVFLFPPKPKDTLMISRTPEVTCVVVDVSHEDPEVKFNWYVDGVEVHNAKTKPREEQYNSTYRVVSVLTVLHQDWLNGKEYKCKVSNKALPAPIEKTISKAKGQPREPQVCTLPPSRDELTKNQVSLSCAVKGFYPSDIAVEWESNGQPENNYKTTPPVLDSDGSFFLVSKLTVDKSRWQQGNVFSCSVMHEALHNHYTQKSLSLSPGK

SEQ ID NO: 27 - protein, 554 aa, Homo sapiens
SGVRLWATRQAMLGQVHEVPEGWLIFVAEQEELYVRVQNGFRKVQLEARTPLPRGTDNEVAALQPPVVQLHDSNPYPRREHPHPTARPWRADDILASPPRLPEPQPYPGAPHHSSYVHLRPARPTSPPAHSHRDFQPVLHLVALNSPLSGGMRGIRGADFQCFQQARAVGLAGTFRAFLSSRLQDLYSIVRRADRAAVPIVNLKDELLFPSWEALFSGSEGPLKPGARIFSFDGKDVLRHPTWPQKSVWHGSDPNGRRLTESYCETWRTEAPSATGQASSLLGGRLLGQSAASCHHAYIVLCIENSFMTASKDDDDDKGGGGSEPKSQDKTHTCPPCPAPELLGGPSVFLFPPKPKDTLMISRTPEVTCVVVDVSHEDPEVKFNWYVDGVEVHNAKTKPREEQYNSTYRVVSVLTVLHQDWLNGKEYKCKVSNKALPAPIEKTISKAKGQPREPQVYTLPPCRDELTKNQVSLWCLVKGFYPSDIAVEWESNGQPENNYKTTPPVLDSDGSFFLYSKLTVDKSRWQQGNVFSCSVMHEALHNHYTQKSLSLSPG

SEQ ID NO: 28 - protein, 232 aa, Homo sapiens
EPKSQDKTHTCPPCPAPELLGGPSVFLFPPKPKDTLMISRTPEVTCVVVDVSHEDPEVKFNWYVDGVEVHNAKTKPREEQYNSTYRVVSVLTVLHQDWLNGKEYKCKVSNKALPAPIEKTISKAKGQPREPQVCTLPPSRDELTKNQVSLSCAVKGFYPSDIAVEWESNGQPENNYKTTPPVLDSDGSFFLVSKLTVDKSRWQQGNVFSCSVMHEALHNHYTQKSLSLSPGK

SEQ ID NO: 29 - protein, 552 aa, Homo sapiens
DKTHTCPPCPAPELLGGPSVFLFPPKPKDTLMISRTPEVTCVVVDVSHEDPEVKFNWYVDGVEVHNAKTKPREEQYNSTYRVVSVLTVLHQDWLNGKEYKCKVSNKALPAPIEKTISKAKGQPREPQVYTLPPCRDELTKNQVSLWCLVKGFYPSDIAVEWESNGQPENNYKTTPPVLDSDGSFFLYSKLTVDKSRWQQGNVFSCSVMHEALHNHYTQKSLSLSPGGGGGSPGSDDDDDKSGVRLWATRQAMLGQVHEVPEGWLIFVAEQEELYVRVQNGFRKVQLEARTPLPRGTDNEVAALQPPVVQLHDSNPYPRREHPHPTARPWRADDILASPPRLPEPQPYPGAPHHSSYVHLRPARPTSPPAHSHRDFQPVLHLVALNSPLSGGMRGIRGADFQCFQQARAVGLAGTFRAFLSSRLQDLYSIVRRADRAAVPIVNLKDELLFPSWEALFSGSEGPLKPGARIFSFDGKDVLRHPTWPQKSVWHGSDPNGRRLTESYCETWRTEAPSATGQASSLLGGRLLGQSAASCHHAYIVLCIENSFMTASK

SEQ ID NO: 30 - protein, 227 aa, Homo sapiens; identical to SEQ ID NO: 26

SEQ ID NO: 31 - protein, 555 aa, Artificial Sequence
  Heterodimeric NC1-Fc, Molecule 1, Chain 1
SGVRLWATRQAMLGQVHEVPEGWLIFVAEQEELYVRVQNGFRKVQLEARTPLPRGTDNEVAALQPPVVQLHDSNPYPRREHPHPTARPWRADDILASPPRLPEPQPYPGAPHHSSYVHLRPARPTSPPAHSHRDFQPVLHLVALNSPLSGGMRGIRGADFQCFQQARAVGLAGTFRAFLSSRLQDLYSIVRRADRAAVPIVNLKDELLFPSWEALFSGSEGPLKPGARIFSFDGKDVLRHPTWPQKSVWHGSDPNGRRLTESYCETWRTEAPSATGQASSLLGGRLLGQSAASCHHAYIVLCIENSFMTASKDDDDDKGGGGSEPKSQDKTHTCPPCPAPELLGGPSVFLFPPKPKDTLMISRTPEVTCVVVDVSHEDPEVKFNWYVDGVEVHNAKTKPREEQYNSTYRVVSVLTVLHQDWLNGKEYKCKVSNKALPAPIEKTISKAKGQPREPQVYTLPPCRDELTKNQVSLWCLVKGFYPSDIAVEWESNGQPENNYKTTPPVLDSDGSFFLYSKLTVDKSRWQQGNVFSCSVMHEALHNHYTQKSLSLSPGK

SEQ ID NO: 32 - protein, 237 aa, Artificial Sequence
  Heterodimeric NC1-Fc, Molecule 1, Chain 2
GGGGSEPKSQDKTHTCPPCPAPELLGGPSVFLFPPKPKDTLMISRTPEVTCVVVDVSHEDPEVKFNWYVDGVEVHNAKTKPREEQYNSTYRVVSVLTVLHQDWLNGKEYKCKVSNKALPAPIEKTISKAKGQPREPQVCTLPPSRDELTKNQVSLSCAVKGFYPSDIAVEWESNGQPENNYKTTPPVLDSDGSFFLVSKLTVDKSRWQQGNVFSCSVMHEALHNHYTQKSLSLSPGK

SEQ ID NO: 33 - protein, 555 aa, Artificial Sequence; identical to SEQ ID NO: 31
  Homodimeric NC1-Fc, Molecule 2, Chain 1

SEQ ID NO: 34 - protein, 555 aa, Artificial Sequence
  Homodimeric NC1-Fc, Molecule 2, Chain 2
SGVRLWATRQAMLGQVHEVPEGWLIFVAEQEELYVRVQNGFRKVQLEARTPLPRGTDNEVAALQPPVVQLHDSNPYPRREHPHPTARPWRADDILASPPRLPEPQPYPGAPHHSSYVHLRPARPTSPPAHSHRDFQPVLHLVALNSPLSGGMRGIRGADFQCFQQARAVGLAGTFRAFLSSRLQDLYSIVRRADRAAVPIVNLKDELLFPSWEALFSGSEGPLKPGARIFSFDGKDVLRHPTWPQKSVWHGSDPNGRRLTESYCETWRTEAPSATGQASSLLGGRLLGQSAASCHHAYIVLCIENSFMTASKDDDDDKGGGGSEPKSQDKTHTCPPCPAPELLGGPSVFLFPPKPKDTLMISRTPEVTCVVVDVSHEDPEVKFNWYVDGVEVHNAKTKPREEQYNSTYRVVSVLTVLHQDWLNGKEYKCKVSNKALPAPIEKTISKAKGQPREPQVCTLPPSRDELTKNQVSLSCAVKGFYPSDIAVEWESNGQPENNYKTTPPVLDSDGSFFLVSKLTVDKSRWQQGNVFSCSVMHEALHNHYTQKSLSLSPGK

SEQ ID NO: 35 - protein, 424 aa, Artificial Sequence
  Heterodimeric Fc-Endostatin, Molecule 3, Chain 1
EPKSQDKTHTCPPCPAPELLGGPSVFLFPPKPKDTLMISRTPEVTCVVVDVSHEDPEVKFNWYVDGVEVHNAKTKPREEQYNSTYRVVSVLTVLHQDWLNGKEYKCKVSNKALPAPIEKTISKAKGQPREPQVYTLPPCRDELTKNQVSLWCLVKGFYPSDIAVEWESNGQPENNYKTTPPVLDSDGSFFLYSKLTVDKSRWQQGNVFSCSVMHEALHNHYTQKSLSLSPGGGGGSGGGGSHSHRDFQPVLHLVALNSPLSGGMRGIRGADFQCFQQARAVGLAGTFRAFLSSRLQDLYSIVRRADRAAVPIVNLKDELLFPSWEALFSGSEGPLKPGARIFSFDGKDVLRHPTWPQKSVWHGSDPNGRRLTESYCETWRTEAPSATGQASSLLGGRLLGQSAASCHHAYIVLCIENSFMTASK

SEQ ID NO: 36 - protein, 241 aa, Artificial Sequence
  Heterodimeric Fc-Endostatin, Molecule 3, Chain 2
EPKSQDKTHTCPPCPAPELLGGPSVFLFPPKPKDTLMISRTPEVTCVVVDVSHEDPEVKFNWYVDGVEVHNAKTKPREEQYNSTYRVVSVLTVLHQDWLNGKEYKCKVSNKALPAPIEKTISKAKGQPREPQVCTLPPSRDELTKNQVSLSCAVKGFYPSDIAVEWESNGQPENNYKTTPPVLDSDGSFFLVSKLTVDKSRWQQGNVFSCSVMHEALHNHYTQKSLSLSPGGGGGSGGGGS

SEQ ID NO: 37 - protein, 539 aa, Artificial Sequence
  Monomeric NC1-Fc, Molecule 4, Chain 1
SGVRLWATRQAMLGQVHEVPEGWLIFVAEQEELYVRVQNGFRKVQLEARTPLPRGTDNEVAALQPPVVQLHDSNPYPRREHPHPTARPWRADDILASPPRLPEPQPYPGAPHHSSYVHLRPARPTSPPAHSHRDFQPVLHLVALNSPLSGGMRGIRGADFQCFQQARAVGLAGTFRAFLSSRLQDLYSIVRRADRAAVPIVNLKDELLFPSWEALFSGSEGPLKPGARIFSFDGKDVLRHPTWPQKSVWHGSDPNGRRLTESYCETWRTEAPSATGQASSLLGGRLLGQSAASCHHAYIVLCIENSFMTASKGGGGSGGGGSAPELLGGPSVFLFPPKPKDTLYITREPEVTCVVVDVSHEDPEVKFNWYVDGVEVHNAKTKPREEQYNSTYRVVSVLTVLHQDWLNGKEYKCKVSNKALPAPIEKTISKAKGQPREPQVYTLPPSRDELTKNQVSLTCLVKGFYPSDIAVEWESNGQPENNYKTTPPVLDSDGSFRLYSKLTVDKSRWQQGNVFSCSVMHEALHNHYTQKSLSLSPGK

SEQ ID NO: 38 - protein, 409 aa, Artificial Sequence
  Monomeric Fc-Endostatin, Molecule 5, Chain 1
APELLGGPSVFLFPPKPKDTLYITREPEVTCVVVDVSHEDPEVKFNWYVDGVEVHNAKTKPREEQYNSTYRVVSVLTVLHQDWLNGKEYKCKVSNKALPAPIEKTISKAKGQPREPQVYTLPPSRDELTKNQVSLTCLVKGFYPSDIAVEWESNGQPENNYKTTPPVLDSDGSFRLYSKLTVDKSRWQQGNVFSCSVMHEALHNHYTQKSLSLSPGGGGGSGGGGSHSHRDFQPVLHLVALNSPLSGGMRGIRGADFQCFQQARAVGLAGTFRAFLSSRLQDLYSIVRRADRAAVPIVNLKDELLFPSWEALFSGSEGPLKPGARIFSFDGKDVLRHPTWPQKSVWHGSDPNGRRLTESYCETWRTEAPSATGQASSLLGGRLLGQSAASCHHAYIVLCIENSFMTASK

SEQ ID NO: 39 - protein, 340 aa, Artificial Sequence
  Cloned Mouse NC1 - PRT
MGWSCIILFLVATATGVHSHHHHHHAGQVRIWATYQTMLDKIREVPEGWLIFVAEREELYVRVRNGFRKVLLEARTALPRGTGNEVAALQPPLVQLHEGSPYTRREYSYSTARPWRADDILANPPRLPDRQPYPGVPHHHSSYVHLPPARPTLSLAHTHQDFQPVLHLVALNTPLSGGMRGIRGADFQCFQQARAVGLSGTFRAFLSSRLQDLYSIVRRADRGSVPIVNLKDEVLSPSWDSLFSGSQGQLQPGARIFSFDGRDVLRHPAWPQKSVWHGSDPSGRRLMESYCETWRTETTGATGQASSLLSGRLLEQKAASCHNSYIVLCIENSFMTSFSK

SEQ ID NO: 40 - DNA, 1047 bp, Artificial Sequence
  Cloned Mouse NC1 – DNA
gaattcccgccgccaccatgggctggtcctgcatcattctgtttctggtggccacagccaccggcgtgcactctcaccatcaccatcatcacgctggccaagtgcggatctgggccacctatcagaccatgctggacaagatcagagaggtgcccgaaggctggctgatcttcgtggccgaacgggaagaactgtacgtcagagtgcggaacggcttcagaaaggtgctgctggaagccagaacagccctgcctagaggcacaggcaatgaagtggctgctctgcagcctcctctggtccaactgcacgagggcagcccttacaccagaagagagtacagctacagcaccgccagaccttggagagccgacgacattctggccaatcctccaagactgcccgacagacagccttatcctggcgtgccacaccaccacagcagctatgttcatctgcctccagccagacctacactgagcctggctcacacccaccaggatttccagcctgtgctgcatctggtggctctgaacacacctctgagcggcggcatgagaggaatcagaggcgccgatttccagtgctttcagcaggccagagccgtgggcctgagcggaacttttagagccttcctgagcagcagactgcaggacctgtacagcattgtgcggagggccgatagaggcagcgtgcccattgtgaacctgaaggacgaggtgctgagcccctcttgggatagcctgtttagcggctctcagggccaactgcaaccaggcgccagaatcttcagcttcgacggcagagatgtgctgagacaccctgcctggcctcagaaatctgtgtggcatggcagcgacccatctggcagacggctgatggaaagctactgcgagacatggcggaccgagacaacaggcgctacaggacaggcaagctctctgctgagtggcagactgctggaacagaaggccgccagctgccacaacagctacatcgtgctgtgcatcgagaacagcttcatgaccagcttcagcaagtgataagctt

SEQ ID NO: 41 - protein, 337 aa, Artificial Sequence
  Cloned Human NC1 – PRT
MGWSCIILFLVATATGVHSHHHHHHSGVRLWATRQAMLGQVHEVPEGWLIFVAEQEELYVRVQNGFRKVQLEARTPLPRGTDNEVAALQPPVVQLHDSNPYPRREHPHPTARPWRADDILASPPRLPEPQPYPGAPHHSSYVHLRPARPTSPPAHSHRDFQPVLHLVALNSPLSGGMRGIRGADFQCFQQARAVGLAGTFRAFLSSRLQDLYSIVRRADRAAVPIVNLKDELLFPSWEALFSGSEGPLKPGARIFSFDGKDVLRHPTWPQKSVWHGSDPNGRRLTESYCETWRTEAPSATGQASSLLGGRLLGQSAASCHHAYIVLCIENSFMTASK

SEQ ID NO: 42 - DNA, 1038 bp, Artificial Sequence
  Cloned Human NC1 – DNA
gaattcccgccgccaccatgggctggtcctgcatcattctgtttctggtggccacagccaccggcgtgcactctcaccatcaccatcatcatagcggcgtgcggctgtgggctacaagacaggctatgctgggacaagtgcacgaggtgccagaaggctggctgatctttgtggccgagcaagaggaactgtacgtgcgggtgcagaacggcttcagaaaggtgcagctggaagccagaacacccctgcctagaggcaccgacaatgaagtggctgctctgcagcctcctgtggtgcagctccacgacagcaacccctatcctagaagagagcaccctcatcctaccgccagaccttggagagccgacgacattctggcctctccacctagactgcctgagcctcagccttatcctggcgctcctcaccacagcagctatgtgcatctgaggcctgccagacctacaagccctcctgctcacagccacagagacttccagcctgtgctgcatctggtggctctgaactctcctctgtccggcggcatgagaggaatcagaggcgccgatttccagtgcttccagcaggccagagctgttggactggccggaaccttcagagccttcctgtctagcagactgcaggacctgtacagcatcgtgcgcagagccgatagagccgccgtgcctatcgtgaacctgaaggacgagctgctgttccctagctgggaagccctgtttagcggctctgagggacctctgaaaccaggcgccagaatcttcagcttcgacggcaaggacgtgctgagacaccctacctggcctcagaaatctgtgtggcacggcagcgaccccaacggaagaaggctgacagagagctactgcgaaacctggcggacagaagccccatctgcaacaggacaggccagctctttgctcggaggtagactgcttggacagagcgccgcctcttgtcaccacgcctatatcgtgctgtgcatcgagaacagcttcatgaccgccagcaagtgataagctt